European Patent Application EP 4 628 104 A1, published October 8, 2025. Title: ANTI-CLDN18.2 ANTIBODY-DRUG CONJUGATE, AND PHARMACEUTICAL COMPOSITION THEREOF AND USE THEREOF. Applicant: SHANGHAI CHIA TAI TIANQING PHARMACEUTICAL TECHNOLOGY DEVELOPMENT CO., LTD. The sequence listing filed with the application follows.

SEQUENCE LISTING (71 sequences)

SEQ ID NO: 1 - protein, 330 aa, synthetic construct [sequence omitted]

SEQ ID NO: 2 - protein, 107 aa, synthetic construct [sequence omitted]

SEQ ID NO: 3 - protein, 5 aa, synthetic construct
  source 1..5: note = HCDR1 of mouse, chimeric, and humanized 28G3
DYLML

SEQ ID NO: 4 - protein, 17 aa, synthetic construct
  source 1..17: note = HCDR2 of mouse and chimeric 28G3
NINPYYGRTTYNLKFKG

SEQ ID NO: 5 - protein, 17 aa, synthetic construct
  source 1..17: note = HCDR2 of hz28G3-1.1, hz28G3-1.3, hz28G3-2.1, and hz28G3-2.3
NINPYYGRTTYALKFKG

SEQ ID NO: 6 - protein, 17 aa, synthetic construct
  source 1..17: note = HCDR2 of hz28G3-1.2, hz28G3-1.4, hz28G3-2.2, and hz28G3-2.4
NINPYYGRTYYALKFQG

SEQ ID NO: 7 - protein, 11 aa, synthetic construct
  source 1..11: note = HCDR3 of mouse, chimeric, and humanized 28G3
DGYSLRNAMDY

SEQ ID NO: 8 - protein, 17 aa, synthetic construct
  source 1..17: note = LCDR1 of mouse, chimeric, and humanized 28G3
KSSQSLFNSGNQKNYLA

SEQ ID NO: 9 - protein, 7 aa, synthetic construct
  source 1..7: note = LCDR2 of mouse, chimeric, and humanized 28G3
GASTRES

SEQ ID NO: 10 - protein, 9 aa, synthetic construct
  source 1..9: note = LCDR3 of mouse, chimeric, and humanized 28G3
QNAHSYPYT

SEQ ID NO: 11 - protein, 120 aa, synthetic construct
  source 1..120: note = VH of mouse and chimeric 28G3
EIQLQQTGPELVKPGASVTISCKTSGYSFTDYLMLWVKQSHGKSLEWIGNINPYYGRTTYNLKFKGKATLTVDRSSSTAYMQLNSLTSEDSAVYYCARDGYSLRNAMDYWGQGTSVTVSS

SEQ ID NO: 12 - protein, 120 aa, synthetic construct
  source 1..120: note = VH of hz28G3-1.1 and hz28G3-2.1
QVQLVQSGAEVKKPGASVKVSCKTSGYSFTDYLMLWVRQAPGQGLEWMGNINPYYGRTTYALKFKGRVTMTVDRSTSTVYMELSSLRSEDTAVYYCARDGYSLRNAMDYWGQGTLVTVSS

SEQ ID NO: 13 - protein, 120 aa, synthetic construct
  source 1..120: note = VH of hz28G3-1.2 and hz28G3-2.2
QVQLVQSGAEVKKPGASVKVSCKASGYTFTDYLMLWVRQAPGQGLEWMGNINPYYGRTYYALKFQGRVTMTVDRSTSTVYMELSSLRSEDTAVYYCARDGYSLRNAMDYWGQGTLVTVSS

SEQ ID NO: 14 - protein, 120 aa, synthetic construct
  source 1..120: note = VH of hz28G3-1.3 and hz28G3-2.3
QVQLVQSGAEVKKPGASVKVSCKTSGYSFTDYLMLWVRQAHGQSLEWMGNINPYYGRTTYALKFKGRVTMTVDRSTSTVYMELSSLRSEDTAVYYCARDGYSLRNAMDYWGQGTLVTVSS

SEQ ID NO: 15 - protein, 120 aa, synthetic construct
  source 1..120: note = VH of hz28G3-1.4 and hz28G3-2.4
QVQLVQSGAEVKKPGASVKVSCKASGYTFTDYLMLWVRQAHGQSLEWMGNINPYYGRTYYALKFQGRVTMTVDRSTSTVYMELSSLRSEDTAVYYCARDGYSLRNAMDYWGQGTLVTVSS

SEQ ID NO: 16 - protein, 113 aa, synthetic construct
  source 1..113: note = VL of mouse and chimeric 28G3
DIVMTQSPYSLSVSTGEKVTMSCKSSQSLFNSGNQKNYLAWYQQKPGQPPKLLIYGASTRESGVPDRFTGSGSGTDFTLTISSVQAEDLALYYCQNAHSYPYTFGGGTKLEIK

SEQ ID NO: 17 - protein, 113 aa, synthetic construct
  source 1..113: note = VL of hz28G3-1.1, hz28G3-1.2, hz28G3-1.3, and hz28G3-1.4
DIVMTQSPDSLAVSLGERATINCKSSQSLFNSGNQKNYLAWYQQKPGQPPKLLIYGASTRESGVPDRFSGSGSGTDFTLTISSLQAEDVAVYYCQNAHSYPYTFGQGTKVEIK

SEQ ID NO: 18 - protein, 113 aa, synthetic construct
  source 1..113: note = VL of hz28G3-2.1, hz28G3-2.2, hz28G3-2.3, and hz28G3-2.4
DIVMTQSPYSLAVSLGERATINCKSSQSLFNSGNQKNYLAWYQQKPGQPPKLLIYGASTRESGVPDRFTGSGSGTDFTLTISSLQAEDVAVYYCQNAHSYPYTFGQGTKVEIK

SEQ ID NO: 19 - protein, 5 aa, synthetic construct
  source 1..5: note = HCDR1 of mouse, chimeric, and humanized 40F6
SYGVY

SEQ ID NO: 20 - protein, 16 aa, synthetic construct
  source 1..16: note = HCDR2 of mouse and chimeric 40F6, hz40F6-1.2, and hz40F6-2.2
VVWAGGNTNYNSALMS

SEQ ID NO: 21 - protein, 16 aa, synthetic construct
  source 1..16: note = HCDR2 of hz40F6-1.1 and hz40F6-2.1
VVWAGGNTNYADSVKG

SEQ ID NO: 22 - protein, 16 aa, synthetic construct
  source 1..16: note = HCDR2 of hz40F6-1.3 and hz40F6-2.3
VVWAGGNTNYADALKG

SEQ ID NO: 23 - protein, 16 aa, synthetic construct
  source 1..16: note = HCDR2 of hz40F6-1.4 and hz40F6-2.4
VVWAGGNTNYNSALKG

SEQ ID NO: 24 - protein, 10 aa, synthetic construct
  source 1..10: note = HCDR3 of mouse, chimeric, and humanized 40F6
DRGRLLAMDY

SEQ ID NO: 25 - protein, 17 aa, synthetic construct
  source 1..17: note = LCDR1 of mouse, chimeric, and humanized 40F6
KSSQSLLNSGNQKNYLA

SEQ ID NO: 26 - protein, 7 aa, synthetic construct
  source 1..7: note = LCDR2 of mouse, chimeric, and humanized 40F6
GASTRES

SEQ ID NO: 27 - protein, 9 aa, synthetic construct
  source 1..9: note = LCDR3 of mouse and chimeric 40F6, hz40F6-1.1, hz40F6-1.2, hz40F6-1.3, and hz40F6-1.4
QNDHFFPFT

SEQ ID NO: 28 - protein, 9 aa, synthetic construct
  source 1..9: note = LCDR3 of hz40F6-2.1, hz40F6-2.2, hz40F6-2.3, and hz40F6-2.4
QNDYFFPFT

SEQ ID NO: 29 - protein, 118 aa, synthetic construct
  source 1..118: note = VH of mouse and chimeric 40F6
QVQLKESGPGLVAPSQSLSITCTVSGFSLTSYGVYWVRQSPGKGLEWLGVVWAGGNTNYNSALMSRLSISKDNSKSQVFLKMNSLQTDDTAMYYCARDRGRLLAMDYWGQGTSVTVSS

SEQ ID NO: 30 - protein, 118 aa, synthetic construct
  source 1..118: note = VH of hz40F6-1.1 and hz40F6-2.1
QVQLVESGGGVVQPGRSLRLSCAASGFTLTSYGVYWVRQAPGKGLEWVAVVWAGGNTNYADSVKGRFTISKDNSKSTLYLQMNSLRAEDTAVYYCARDRGRLLAMDYWGQGTLVTVSS

SEQ ID NO: 31 - protein, 118 aa, synthetic construct
  source 1..118: note = VH of hz40F6-1.2 and hz40F6-2.2
QVQLVESGGGVVQPGRSLRLSCAASGFTLTSYGVYWVRQAPGKGLEWVAVVWAGGNTNYNSALMSRFTISKDNSKSTLYLQMNSLRAEDTAVYYCARDRGRLLAMDYWGQGTLVTVSS

SEQ ID NO: 32 - protein, 118 aa, synthetic construct
  source 1..118: note = VH of hz40F6-1.3 and hz40F6-2.3
QVQLVESGGGVVQPGRSLRLSCAASGFTLTSYGVYWVRQAPGKGLEWVAVVWAGGNTNYADALKGRFTISKDNSKSTLYLQMNSLRAEDTAVYYCARDRGRLLAMDYWGQGTLVTVSS

SEQ ID NO: 33 - protein, 118 aa, synthetic construct
  source 1..118: note = VH of hz40F6-1.4 and hz40F6-2.4
QVQLVESGGGVVQPGRSLRLSCTVSGFTLTSYGVYWVRQAPGKGLEWVAVVWAGGNTNYNSALKGRFTISKDNSKSTLYLQMNSLRAEDTAVYYCARDRGRLLAMDYWGQGTLVTVSS

SEQ ID NO: 34 - protein, 113 aa, synthetic construct
  source 1..113: note = VL of mouse and chimeric 40F6
DVVMTQSPSSLSVSAGEKVTMSCKSSQSLLNSGNQKNYLAWYQQKPGQPPKLLIYGASTRESGVPDRFTGSGSGTDFTLTISSVQAEDLAVYYCQNDHFFPFTFGSGTKLEIK

SEQ ID NO: 35 - protein, 113 aa, synthetic construct
  source 1..113: note = VL of hz40F6-1.1, hz40F6-1.2, hz40F6-1.3, and hz40F6-1.4
DIVMTQSPDSLAVSLGERATINCKSSQSLLNSGNQKNYLAWYQQKPGQPPKLLIYGASTRESGVPDRFTGSGSGTDFTLTISSLQAEDVAVYYCQNDHFFPFTFGQGTKVEIK

SEQ ID NO: 36 - protein, 113 aa, synthetic construct
  source 1..113: note = VL of hz40F6-2.1, hz40F6-2.2, hz40F6-2.3, and hz40F6-2.4
DIVMTQSPDSLAVSLGERATINCKSSQSLLNSGNQKNYLAWYQQKPGQPPKLLIYGASTRESGVPDRFSGSGSGTDFTLTISSLQAEDVAVYYCQNDYFFPFTFGQGTKVEIK

SEQ ID NO: 37 - protein, 5 aa, synthetic construct
  source 1..5: note = HCDR1 of mouse and chimeric 34G6
SYGVH

SEQ ID NO: 38 - protein, 16 aa, synthetic construct
  source 1..16: note = HCDR2 of mouse and chimeric 34G6
VIWSDGSTTYNSALKS

SEQ ID NO: 39 - protein, 10 aa, synthetic construct
  source 1..10: note = HCDR3 of mouse and chimeric 34G6
HAYYGNSFDY

SEQ ID NO: 40 - protein, 17 aa, synthetic construct
  source 1..17: note = LCDR1 of mouse and chimeric 34G6
KSSQSLLNSGNQKSYLT

SEQ ID NO: 41 - protein, 7 aa, synthetic construct
  source 1..7: note = LCDR2 of mouse and chimeric 34G6
WASTRES

SEQ ID NO: 42 - protein, 9 aa, synthetic construct
  source 1..9: note = LCDR3 of mouse and chimeric 34G6
QNVYIFPLT

SEQ ID NO: 43 - protein, 118 aa, synthetic construct
  source 1..118: note = VH of mouse and chimeric 34G6
QVQLKESGPDLVAPSQSLSITCTVSGFSLTSYGVHWVRQPPGKGLEWLVVIWSDGSTTYNSALKSRLSISKDNSKSQVFLKMNSLQTDDTAIYYCARHAYYGNSFDYWGQGTTLTVSS

SEQ ID NO: 44 - protein, 113 aa, synthetic construct
  source 1..113: note = VL of mouse and chimeric 34G6
DIVMTQSPSSLTVTAGEKVTMSCKSSQSLLNSGNQKSYLTWYQQKPGQPPKLLIYWASTRESGVPDRFTGSGSGTDFTLTISSVQAEDLAVYYCQNVYIFPLTFGAGTKLELK

SEQ ID NO: 45 - protein, 5 aa, synthetic construct
  source 1..5: note = HCDR1 of mouse and chimeric 10D8
NYGMN

SEQ ID NO: 46 - protein, 17 aa, synthetic construct
  source 1..17: note = HCDR2 of mouse and chimeric 10D8
WININTGEPRYAEEFKG

SEQ ID NO: 47 - protein, 9 aa, synthetic construct
  source 1..9: note = HCDR3 of mouse and chimeric 10D8
YGYGNSFPY

SEQ ID NO: 48 - protein, 17 aa, synthetic construct
  source 1..17: note = LCDR1 of mouse and chimeric 10D8
KSSQSLLNSGNQRNYLT

SEQ ID NO: 49 - protein, 7 aa, synthetic construct
  source 1..7: note = LCDR2 of mouse and chimeric 10D8
WASTRES

SEQ ID NO: 50 - protein, 9 aa, synthetic construct
  source 1..9: note = LCDR3 of mouse and chimeric 10D8
QNDYSYPLT

SEQ ID NO: 51 - protein, 118 aa, synthetic construct
  source 1..118: note = VH of mouse and chimeric 10D8
QIQLAQSGPELKKPGETVKVSCKASGYTFKNYGMNWVKQAPGKGLKWMGWININTGEPRYAEEFKGRIAFSLETSASTAYLLINNLKNEDTATYFCARYGYGNSFPYWGQGTLVTVSA

SEQ ID NO: 52 - protein, 113 aa, synthetic construct
  source 1..113: note = VL of mouse and chimeric 10D8
DIVMTQSPSSLTVTVGEKVTMSCKSSQSLLNSGNQRNYLTWYQQKPGQPPKLLIYWASTRESGVPDRFTGSGSGTAFTLTVSSVQAEDLAVYYCQNDYSYPLTFGAGTKLEMK

SEQ ID NO: 53 - protein, 5 aa, synthetic construct
  source 1..5: note = HCDR1 of mouse and chimeric 22F12
SYGVY

SEQ ID NO: 54 - protein, 16 aa, synthetic construct
  source 1..16: note = HCDR2 of mouse and chimeric 22F12
VIWAGGSTNYNSALMS

SEQ ID NO: 55 - protein, 10 aa, synthetic construct
  source 1..10: note = HCDR3 of mouse and chimeric 22F12
DRGRLLSMDY

SEQ ID NO: 56 - protein, 17 aa, synthetic construct
  source 1..17: note = LCDR1 of mouse and chimeric 22F12
RSSQSLLNSGNQKNYLA

SEQ ID NO: 57 - protein, 7 aa, synthetic construct
  source 1..7: note = LCDR2 of mouse and chimeric 22F12
GASTRES

SEQ ID NO: 58 - protein, 9 aa, synthetic construct
  source 1..9: note = LCDR3 of mouse and chimeric 22F12
QNVHFFPFT

SEQ ID NO: 59 - protein, 118 aa, synthetic construct
  source 1..118: note = VH of mouse and chimeric 22F12
QVQLKESGPGLVAPSQSLSITCTVSGFSLTSYGVYWVRQPPGKGLEWLGVIWAGGSTNYNSALMSRLSINKDNSKSQVFLKMNSLQTDDTAMYYCARDRGRLLSMDYWGQGTSVTVSS

SEQ ID NO: 60 - protein, 113 aa, synthetic construct
  source 1..113: note = VL of mouse and chimeric 22F12
DIVMTQSPSSLSVSAGEKVTMSCRSSQSLLNSGNQKNYLAWYQQKPGQPPKLLIYGASTRESGVPDRFTGSGSGTDFTLTIGSVQAEDLAVYYCQNVHFFPFTFGSGTKLEIK

SEQ ID NO: 61 - protein, 450 aa, synthetic construct
  source 1..450: note = Heavy chain of hz28G3-1.1
QVQLVQSGAEVKKPGASVKVSCKTSGYSFTDYLMLWVRQAPGQGLEWMGNINPYYGRTTYALKFKGRVTMTVDRSTSTVYMELSSLRSEDTAVYYCARDGYSLRNAMDYWGQGTLVTVSSASTKGPSVFPLAPSSKSTSGGTAALGCLVKDYFPEPVTVSWNSGALTSGVHTFPAVLQSSGLYSLSSVVTVPSSSLGTQTYICNVNHKPSNTKVDKKVEPKSCDKTHTCPPCPAPELLGGPSVFLFPPKPKDTLMISRTPEVTCVVVDVSHEDPEVKFNWYVDGVEVHNAKTKPREEQYNSTYRVVSVLTVLHQDWLNGKEYKCKVSNKALPAPIEKTISKAKGQPREPQVYTLPPSRDELTKNQVSLTCLVKGFYPSDIAVEWESNGQPENNYKTTPPVLDSDGSFFLYSKLTVDKSRWQQGNVFSCSVMHEALHNHYTQKSLSLSPGK

SEQ ID NO: 62 - protein, 220 aa, synthetic construct
  source 1..220: note = Light chain of hz28G3-1.1
DIVMTQSPDSLAVSLGERATINCKSSQSLFNSGNQKNYLAWYQQKPGQPPKLLIYGASTRESGVPDRFSGSGSGTDFTLTISSLQAEDVAVYYCQNAHSYPYTFGQGTKVEIKRTVAAPSVFIFPPSDEQLKSGTASVVCLLNNFYPREAKVQWKVDNALQSGNSQESVTEQDSKDSTYSLSSTLTLSKADYEKHKVYACEVTHQGLSSPVTKSFNRGEC

SEQ ID NO: 63 - protein, 450 aa, synthetic construct
  source 1..450: note = Heavy chain of hz28G3-1.3
QVQLVQSGAEVKKPGASVKVSCKTSGYSFTDYLMLWVRQAHGQSLEWMGNINPYYGRTTYALKFKGRVTMTVDRSTSTVYMELSSLRSEDTAVYYCARDGYSLRNAMDYWGQGTLVTVSSASTKGPSVFPLAPSSKSTSGGTAALGCLVKDYFPEPVTVSWNSGALTSGVHTFPAVLQSSGLYSLSSVVTVPSSSLGTQTYICNVNHKPSNTKVDKKVEPKSCDKTHTCPPCPAPELLGGPSVFLFPPKPKDTLMISRTPEVTCVVVDVSHEDPEVKFNWYVDGVEVHNAKTKPREEQYNSTYRVVSVLTVLHQDWLNGKEYKCKVSNKALPAPIEKTISKAKGQPREPQVYTLPPSRDELTKNQVSLTCLVKGFYPSDIAVEWESNGQPENNYKTTPPVLDSDGSFFLYSKLTVDKSRWQQGNVFSCSVMHEALHNHYTQKSLSLSPGK

SEQ ID NO: 64 - protein, 220 aa, synthetic construct; identical to SEQ ID NO: 62
  source 1..220: note = Light chain of hz28G3-1.3

SEQ ID NO: 65 - protein, 261 aa, Homo sapiens
MAVTACQGLGFVVSLIGIAGIIAATCMDQWSTQDLYNNPVTAVFNYQGLWRSCVRESSGFTECRGYFTLLGLPAMLQAVRALMIVGIVLGAIGLLVSIFALKCIRIGSMEDSAKANMTLTSGIMFIVSGLCAIAGVSVFANMLVTNFWMSTANMYTGMGGMVQTVQTRYTFGAALFVGWVAGGLTLIGGVMMCIACRGLAPEETNYKAVSYHASGHSVAYKPGGFKASTGFGSNTKNKKIYDGGARTEDEVQSYPSKHDYV

SEQ ID NO: 66 - protein, 261 aa, Homo sapiens
MSTTTCQVVAFLLSILGLAGCIAATGMDMWSTQDLYDNPVTSVFQYEGLWRSCVRQSSGFTECRPYFTILGLPAMLQAVRALMIVGIVLGAIGLLVSIFALKCIRIGSMEDSAKANMTLTSGIMFIVSGLCAIAGVSVFANMLVTNFWMSTANMYTGMGGMVQTVQTRYTFGAALFVGWVAGGLTLIGGVMMCIACRGLAPEETNYKAVSYHASGHSVAYKPGGFKASTGFGSNTKNKKIYDGGARTEDEVQSYPSKHDYV

SEQ ID NO: 67 - protein, 448 aa, synthetic construct
  source 1..448: note = Heavy chain of 15F9
QVQLVQSGSELKKPGASVKVSCKASGYTFTNYGINWVRQAPGQGLEWMGWINPNTGETTYAEEFKGRFVFSLDTSVSTAYLQISSLKAEDTAVYFCARLYYGNRFDSWGQGTLVTVSSASTKGPSVFPLAPSSKSTSGGTAALGCLVKDYFPEPVTVSWNSGALTSGVHTFPAVLQSSGLYSLSSVVTVPSSSLGTQTYICNVNHKPSNTKVDKKVEPKSCDKTHTCPPCPAPELLGGPSVFLFPPKPKDTLMISRTPEVTCVVVDVSHEDPEVKFNWYVDGVEVHNAKTKPREEQYNSTYRVVSVLTVLHQDWLNGKEYKCKVSNKALPAPIEKTISKAKGQPREPQVYTLPPSRDELTKNQVSLTCLVKGFYPSDIAVEWESNGQPENNYKTTPPVLDSDGSFFLYSKLTVDKSRWQQGNVFSCSVMHEALHNHYTQKSLSLSPGK

SEQ ID NO: 68 - protein, 220 aa, synthetic construct
  source 1..220: note = Light chain of 15F9
DIVMTQSPDSLAVSLGERATINCKSSQSLLNSGNQRNYLTWYQQKPGQPPKLLIYWASTRESGVPDRFSGSGSGTDFTLTISSLQAEDVAVYYCQNAYYYPLTFGGGTKVEIKRTVAAPSVFIFPPSDEQLKSGTASVVCLLNNFYPREAKVQWKVDNALQSGNSQESVTEQDSKDSTYSLSSTLTLSKADYEKHKVYACEVTHQGLSSPVTKSFNRGEC

SEQ ID NO: 69 - protein, 17 aa, synthetic construct
  source 1..17: note = HCDR2 of mouse, chimeric, and humanized 28G3
  VARIANT 10: note = X = T or Y
  VARIANT 12: note = X = N or A
  VARIANT 16: note = X = K or Q
NINPYYGRTXYXLKFXG

SEQ ID NO: 70 - protein, 16 aa, synthetic construct
  source 1..16: note = HCDR2 of mouse, chimeric, and humanized 40F6
  VARIANT 11: note = X = N or A
  VARIANT 12: note = X = S or D
  VARIANT 13: note = X = A or S
  VARIANT 14: note = X = L or V
  VARIANT 15: note = X = M or K
  VARIANT 16: note = X = S or G
VVWAGGNTNYXXXXXX

SEQ ID NO: 71 - protein, 9 aa, synthetic construct
  source 1..9: note = LCDR3 of mouse, chimeric, and humanized 40F6
  VARIANT 4: note = X = H or Y
QNDXFFPFT